European Patent Application EP 4 345 113 A1, published April 3, 2024. Title: Przeciwciało anty-HER2, cząsteczka kwasu nukleinowego kodująca region zmienny tego przeciwciała, sposób wykrywania HER2 w próbce biologicznej, test immuno-enzymatyczny ELISA oraz zastosowanie przeciwciała anty-HER2 lub jego fragmentów. Applicant: SDS OPTIC S.A. The sequence listing filed with the application follows.

SEQUENCE LISTING (40 sequences)

SEQ ID NO: 1 - protein, 8 aa, unidentified
GYSFTGYN

SEQ ID NO: 2 - protein, 8 aa, unidentified
GYSFTDYN

SEQ ID NO: 3 - protein, 7 aa, unidentified
IDPNYGT

SEQ ID NO: 4 - protein, 8 aa, unidentified
IDHYNGNT

SEQ ID NO: 5 - protein, 13 aa, unidentified
ARRKVNYEAWFAF

SEQ ID NO: 6 - protein, 11 aa, unidentified
ARHYDYGAMDY

SEQ ID NO: 7 - protein, 10 aa, unidentified
ESVDSYGNSF

SEQ ID NO: 8 - protein, 6 aa, unidentified
QNVGTN

SEQ ID NO: 9-10 - skipped (2 entries)

SEQ ID NO: 11 - protein, 9 aa, unidentified
QQSNEDPFT

SEQ ID NO: 12 - protein, 9 aa, unidentified
QHYYIYPLT

SEQ ID NO: 13 - protein, 119 aa, unidentified
EVQLQQSGPELEKPGASVKISCKASGYSFTGYNMNWVKQSNGKSLEWIGTIDPNYGTSYNQKFKGKATLTVDKSSSTAYMHLKSLTSEDSSVYYCARRKVNYEAWFAFWGQGTLVTVSA

SEQ ID NO: 14 - protein, 118 aa, unidentified
EIQLQQSGPELVKPGASVRVSCKASGYSFTDYNMYWVRQSQGESLEWIGYIDHYNGNTGYNQKFRDKATLTVDKASSTAFMHLNSLTSEDSAVYYCARHYDYGAMDYWGQGTSVTVSS

SEQ ID NO: 15 - protein, 112 aa, unidentified
DIVLTQSPASLAVSLGQRATISCRASESVDSYGNSFMHWYQQKPGQPPKLLIYRASNLESGIPARFSGSGSRTDFTLTINPVEADDVATYYCQQSNEDPFTFGSGTKLEIKR

SEQ ID NO: 16 - protein, 108 aa, unidentified
DIVMTQSQKFMSTSVGDRVSVTCKASQNVGTNVAWYQQKPGQSPKALIYSASYRYSGVPDRFTGSGSGTDFTLTISTVQSEDLAEYFCQHYYIYPLTFGAGTKLELKR

SEQ ID NO: 17 - DNA, 24 bp, unidentified
  source 1..24: mol_type = unassigned DNA
ggttactcattcactggctacaac

SEQ ID NO: 18 - DNA, 24 bp, unidentified
  source 1..24: mol_type = unassigned DNA
ggttactcattcactgactacaac

SEQ ID NO: 19 - DNA, 24 bp, unidentified
  source 1..24: mol_type = unassigned DNA
attgatcctaactatggtggtact

SEQ ID NO: 20 - DNA, 24 bp, unidentified
  source 1..24: mol_type = unassigned DNA
attgatcattacaatggaaatact

SEQ ID NO: 21 - DNA, 39 bp, unidentified
  source 1..39: mol_type = unassigned DNA
gcaagacggaaggttaactacgaggcctggtttgctttc

SEQ ID NO: 22 - DNA, 33 bp, unidentified
  source 1..33: mol_type = unassigned DNA
gcaagacactacgactacggtgctatggactac

SEQ ID NO: 23 - DNA, 30 bp, unidentified
  source 1..30: mol_type = unassigned DNA
gaaagtgttgatagttatggcaatagtttt

SEQ ID NO: 24 - DNA, 18 bp, unidentified
  source 1..18: mol_type = unassigned DNA
cagaatgtgggtactaat

SEQ ID NO: 25-26 - skipped (2 entries)

SEQ ID NO: 27 - DNA, 27 bp, unidentified
  source 1..27: mol_type = unassigned DNA
cagcaaagtaatgaggatccattcacg

SEQ ID NO: 28 - DNA, 27 bp, unidentified
  source 1..27: mol_type = unassigned DNA
cagcattattacatctatccgctcacg

SEQ ID NO: 29 - protein, 474 aa, unidentified
MGWTWIFILILSVTTGVHSEVQLQQSGPELEKPGASVKISCKASGYSFTGYNMNWVKQSNGKSLEWIGTIDPNYGTSYNQKFKGKATLTVDKSSSTAYMHLKSLTSEDSSVYYCARRKVNYEAWFAFWGQGTLVTVSAAKTTPPSVYPLAPGCGDTTGSSVTLGCLVKGYFPESVTVTWNSGSLSSSVHTFPALLQSGLYTMSSSVTVPSSTWPSQTVTCSVAHPASSTTVDKKLEPSGPISTINPCPPCKECHKCPAPNLEGGPSVFIFPPNIKDVLMISLTPKVTCVVVDVSEDDPDVQISWFVNNVEVHTAQTQTHREDYNSTIRVVSTLPIQHQDWMSGKEFKCKVNNKDLPSPIERTISKIKGLVRAPQVYILPPPAEQLSRKDVSLTCLVVGFNPGDISVEWTSNGHTEENYKDTAPVLDSDGSYFIYSKLNMKTSKWEKTDSFSCNVRHEGLKNYYLKKTISRTPGK

SEQ ID NO: 30 - protein, 473 aa, unidentified
MEWSWIFLFLLSGTTGVHSEIQLQQSGPELVKPGASVRVSCKASGYSFTDYNMYWVRQSQGESLEWIGYIDHYNGNTGYNQKFRDKATLTVDKASSTAFMHLNSLTSEDSAVYYCARHYDYGAMDYWGQGTSVTVSSAKTTPPSVYPLAPGCGDTTGSSVTLGCLVKGYFPESVTVTWNSGSLSSSVHTFPALLQSGLYTMSSSVTVPSSTWPSQTVTCSVAHPASSTTVDKKLEPSGPISTINPCPPCKECHKCPAPNLEGGPSVFIFPPNIKDVLMISLTPKVTCVVVDVSEDDPDVQISWFVNNVEVHTAQTQTHREDYNSTIRVVSTLPIQHQDWMSGKEFKCKVNNKDLPSPIERTISKIKGLVRAPQVYILPPPAEQLSRKDVSLTCLVVGFNPGDISVEWTSNGHTEENYKDTAPVLDSDGSYFIYSKLNMKTSKWEKTDSFSCNVRHEGLKNYYLKKTISRTPGK

SEQ ID NO: 31 - protein, 238 aa, unidentified
METDTLLLWVLLLWVPGSTGDIVLTQSPASLAVSLGQRATISCRASESVDSYGNSFMHWYQQKPGQPPKLLIYRASNLESGIPARFSGSGSRTDFTLTINPVEADDVATYYCQQSNEDPFTFGSGTKLEIKRADAAPTVSIFPPSSEQLTSGGASVVCFLNNFYPKDINVKWKIDGSERQNGVLNSWTDQDSKDSTYSMSSTLTLTKDEYERHNSFTCEATHKTSTSPIVKSFNRNEC

SEQ ID NO: 32 - protein, 234 aa, unidentified
MESQTQVFVYMLLWLSGVDGDIVMTQSQKFMSTSVGDRVSVTCKASQNVGTNVAWYQQKPGQSPKALIYSASYRYSGVPDRFTGSGSGTDFTLTISTVQSEDLAEYFCQHYYIYPLTFGAGTKLELKRADAAPTVSIFPPSSEQLTSGGASVVCFLNNFYPKDINVKWKIDGSERQNGVLNSWTDQDSKDSTYSMSSTLTLTKDEYERHNSYTCEATHKTSTSPIVKSFNRNEC

SEQ ID NO: 33 - DNA, 1532 bp, unidentified
  source 1..1532: mol_type = unassigned DNA
atgggatggacctggatctttattttaatcctgtcagtaactacaggtgtccactctgaggtccagctgcagcagtctggacctgagctggagaagcctggcgcttcagtgaagatatcctgcaaggcttctggttactcattcactggctacaacatgaactgggtgaagcagagcaatggaaagagtcttgagtggattggaactattgatcctaactatggtggtactcttctggttactcattcactggctacaacatgaactgggtgaagcagagcaatggaaagagtcttgagtggattggaactattgatcctaactatggtggtactagctacaaccagaagttcaagggcaaggccacattgactgtagacaaatcctccagcacagcctacatgcacctcaagagcctgacatctgaggactcttcagtctattactgtgcaagacggaaggttaactacgaggcctggtttgctttctggggccaagggactctggtcactgtctctgcagccaaaacaacacccccatcagtctatccactggcccctgggtgtggagatacaactggttcctccgtgactctgggatgcctggtcaagggctacttccctgagtcagtgactgtgacttggaactctggatccctgtccagcagtgtgcacaccttcccagctctcctgcagtctggactctacactatgagcagctcagtgactgtcccctccagcacctggccaagtcagaccgtcacctgcagcgttgctcacccagccagcagcaccacggtggacaaaaaacttgagcccagcgggcccatttcaacaatcaacccctgtcctccatgcaaggagtgtcacaaatgcccagctcctaacctcgagggtggaccatccgtcttcatcttccctccaaatatcaaggatgtactcatgatctccctgacacccaaggtcacgtgtgtggtggtggatgtgagcgaggatgacccagacgtccagatcagctggtttgtgaacaacgtggaagtacacacagctcagacacaaacccatagagaggattacaacagtactatccgggtggtcagcaccctccccatccagcaccaggactggatgagtggcaaggagttcaaatgcaaggtcaacaacaaagacctcccatcacccatcgagagaaccatctcaaaaattaaagggctagtcagagctccacaagtatacatcttgccgccaccagcagagcagttgtccaggaaagatgtcagtctcacttgcctggtcgtgggcttcaaccctggagacatcagtgtggagtggaccagcaatgggcatacagaggagaactacaaggacaccgcaccagtcctggactctgacggttcttacttcatatatagcaagctcaatatgaaaacaagcaagtgggagaaaacagattccttctcatgcaacgtgagacacgagggtctaaaaaattactacctgaagaagaccatctcccggactccgggtaaatga

SEQ ID NO: 34 - DNA, 1452 bp, unidentified
  source 1..1452: mol_type = unassigned DNA
atggaatggagctggatctttctcttcctcctgtcaggaactacaggtgtccactctgagatccagctgcagcagtctggacctgagctggtgaagcctggggcttcagtgagggtatcctgcaaggcttctggttactcattcactgactacaacatgtactgggtgaggcagagccaaggagagagccttgagtggattggatatattgatcattacaatggaaatactggctataaccagaagttcagggacaaggccacattgactgttgacaaggcctccagcacagccttcatgcatctcaacagcctgacatctgaggactctgcagtctattactgtgcaagacactacgactacggtgctatggactactggggtcaaggaacctcagtcaccgtctcctcaggtcaaggaacctcagtcaccgtctcctcagccaaaacaacacccccatcagtctatccactggcccctgggtgtggagatacaactggttcctccgtgactctgggatgcctggtcaagggctacttccctgagtcagtgactgtgacttggaactctggatccctgtccagcagtgtgcacaccttcccagctctcctgcagtctggactctacactatgagcagctcagtgactgtcccctccagcacctggccaagtcagaccgtcacctgcagcgttgctcacccagccagcagcaccacggtggacaaaaaacttgagcccagcgggcccatttcaacaatcaacccctgtcctccatgcaaggagtgtcacaaatgcccagctcctaacctcgagggtggaccatccgtcttcatcttccctccaaatatcaaggatgtactcatgatctccctgacacccaaagtcacgtgtgtggtggtggatgtgagcgaggatgacccagacgtccagatcagctggtttgtgaacaacgtggaagtacacacagctcagacacaaacccatagagaggattacaacagtactatccgggtggtcagcaccctccccatccagcaccaggactggatgagtggcaaggagttcaaatgcaaggtcaacaacaaagacctcccatcacccatcgagagaaccatctcaaaaattaaagggctagtcagagctccacaagtatacatcttgccgccaccagcagagcagttgtccaggaaagatgtcagtctcacttgcctggtcgtgggcttcaaccctggagacatcagtgtggagtggaccagcaatgggcatacagaggagaactacaaggacaccgcaccagtcctggactctgacggttcttacttcatatatagcaagctcaatatgaaaacaagcaagtgggagaaaacagattccttctcatgcaacgtgagacacgagggtctgaaaaattactacctgaagaagaccatctcccggactccgggtaaatga

SEQ ID NO: 35 - DNA, 717 bp, unidentified
  source 1..717: mol_type = unassigned DNA
atggagacagacacactcctgctatgggtgctgctgctctgggttccaggttccacaggtgacattgtgctgacccaatctccagcttctttggctgtgtctctagggcagagggccaccatatcctgcagagccagtgaaagtgttgatagttatggcaatagttttatgcattggtaccagcagaaaccaggacagccacccaaactcctcatctatcgtgcatccaacctagaatctgggatccctgccaggttcagtggcagtgggtctaggacagacttcaccctcaccattaatcctgtggaggctgatgatgttgcaacctattactgtcagcaaagtaatgaggatccattcacgttcggctcggggacaaagttggaaataaaacgggctgatgctgcaccaactgtatccatcttcccaccatccagtgagcagttaacatctggaggtgcctcagtcgtgtgcttcttgaacaacttctaccccaaagacatcaatgtcaagtggaagattgatggcagtgaacgacaaaatggcgtcctgaacagttggactgatcaggacagcaaagacagcacctacagcatgagcagcaccctcacgttgaccaaggacgagtatgaacgacataacagctttacctgtgaggccactcacaagacatcaacttcacccattgtcaagagcttcaacaggaatgagtgttag

SEQ ID NO: 36 - DNA, 705 bp, unidentified
  source 1..705: mol_type = unassigned DNA
atggagtcacagactcaggtctttgtatacatgttgctgtggttgtctggtgttgatggagacattgtgatgacccagtctcaaaaattcatgtccacatcagtaggagacagggtcagcgtcacctgcaaggccagtcagaatgtgggtactaatgtagcctggtatcaacagaaaccagggcaatctcctaaagcactgatttattcggcatcctaccggtacagtggagtccctgatcgcttcacaggcagtggatctgggacagatttcactctcaccatcagcactgtgcagtctgaagacttggcagagtatttctgtcagcattattacatctatccgctcacgttcggtgctgggaccaagctggagctgaaacgggctgatgctgcaccaactgtatccatcttcccaccatccagtgagcagttaacatctggaggtgcctcagtcgtgtgcttcttgaacaacttctaccccaaagacatcaatgtcaagtggaagattgatggcagtgaacgacaaaatggcgtcctgaacagttggactgatcaggacagcaaagacagcacctacagcatgagcagcaccctcacgttgaccaaggacgagtatgaacgacataacagctatacctgtgaggccactcacaagacatcaacttcacccattgtcaagagcttcaacaggaatgagtgttag

SEQ ID NO: 37 - DNA, 464 bp, unidentified
  source 1..464: mol_type = unassigned DNA
gaggtccagctgcagcagtctggacctgagctggagaagcctggcgcttcagtgaagatatcctgcaaggcttctggttactcattcactggctacaacatgaactgggtgaagcagagcaatggaaagagtcttgagtggattggaactattgatcctaactatggtggtactcttctggttactcattcactggctacaacatgaactgggtgaagcagagcaatggaaagagtcttgagtggattggaactattgatcctaactatggtggtactagctacaaccagaagttcaagggcaaggccacattgactgtagacaaatcctccagcacagcctacatgcacctcaagagcctgacatctgaggactcttcagtctattactgtgcaagacggaaggttaactacgaggcctggtttgctttctggggccaagggactctggtcactgtctctgca

SEQ ID NO: 38 - DNA, 354 bp, unidentified
  source 1..354: mol_type = unassigned DNA
gagatccagctgcagcagtctggacctgagctggtgaagcctggggcttcagtgagggtatcctgcaaggcttctggttactcattcactgactacaacatgtactgggtgaggcagagccaaggagagagccttgagtggattggatatattgatcattacaatggaaatactggctataaccagaagttcagggacaaggccacattgactgttgacaaggcctccagcacagccttcatgcatctcaacagcctgacatctgaggactctgcagtctattactgtgcaagacactacgactacggtgctatggactactggggtcaaggaacctcagtcaccgtctcctca

SEQ ID NO: 39 - DNA, 336 bp, unidentified
  source 1..336: mol_type = unassigned DNA
gacattgtgctgacccaatctccagcttctttggctgtgtctctagggcagagggccaccatatcctgcagagccagtgaaagtgttgatagttatggcaatagttttatgcattggtaccagcagaaaccaggacagccacccaaactcctcatctatcgtgcatccaacctagaatctgggatccctgccaggttcagtggcagtgggtctaggacagacttcaccctcaccattaatcctgtggaggctgatgatgttgcaacctattactgtcagcaaagtaatgaggatccattcacgttcggctcggggacaaagttggaaataaaacgg

SEQ ID NO: 40 - DNA, 324 bp, unidentified
  source 1..324: mol_type = unassigned DNA
gacattgtgatgacccagtctcaaaaattcatgtccacatcagtaggagacagggtcagcgtcacctgcaaggccagtcagaatgtgggtactaatgtagcctggtatcaacagaaaccagggcaatctcctaaagcactgatttattcggcatcctaccggtacagtggagtccctgatcgcttcacaggcagtggatctgggacagatttcactctcaccatcagcactgtgcagtctgaagacttggcagagtatttctgtcagcattattacatctatccgctcacgttcggtgctgggaccaagctggagctgaaacgg